European Patent Application EP 4 260 857 A1, published October 18, 2023. Title: Composition for use in improving hair quality. Applicant: Dr. Cherry Inc. The sequence listing filed with the application follows.

SEQUENCE LISTING (27 sequences)

SEQ ID NO: 1 - DNA, 22 bp, Artificial Sequence
  Probe for rat RplP0
cctgtcttccctgggcatcacg

SEQ ID NO: 2 - DNA, 17 bp, Artificial Sequence
  Primer-1 for rat RplP0
caatccctgacgcaccg

SEQ ID NO: 3 - DNA, 20 bp, Artificial Sequence
  Primer-2 for rat RplP0
tgtctgctcccacaatgaag

SEQ ID NO: 4 - DNA, 24 bp, Artificial Sequence
  Probe for rat Cd34
tccctggaagtaccagccactact

SEQ ID NO: 5 - DNA, 23 bp, Artificial Sequence
  Primer-1 for rat CD34
ggagtatttccaccagttcctac

SEQ ID NO: 6 - DNA, 21 bp, Artificial Sequence
  Primer-2 for rat CD34
gatggctggtgtggtcttatt

SEQ ID NO: 7 - DNA, 24 bp, Artificial Sequence
  Prove for rat PPARG
cctgggcggtctccactgagaata

SEQ ID NO: 8 - DNA, 23 bp, Artificial Sequence
  Primer-1 for rat PPARG
gaattagatgacagtgacttggc

SEQ ID NO: 9 - DNA, 20 bp, Artificial Sequence
  Primer-2 for rat PPARG
agcaggttgtcttggatgtc

SEQ ID NO: 10 - DNA, 25 bp, Artificial Sequence
  Probe for rat CD163
acccaacggcttacagtttcctcaa

SEQ ID NO: 11 - DNA, 21 bp, Artificial Sequence
  Primer-1 for rat CD163
tcatccgtcttcgaatccatc

SEQ ID NO: 12 - DNA, 21 bp, Artificial Sequence
  Primer-2 for rat CD163
tctcattgccttcctcttgtg

SEQ ID NO: 13 - DNA, 27 bp, Artificial Sequence
  Probe for rat CD68
ctctgatgtcggtcctgtttgaatcca

SEQ ID NO: 14 - DNA, 20 bp, Artificial Sequence
  Primer-1 for rat CD68
tgagaatgtccactgtgctg

SEQ ID NO: 15 - DNA, 22 bp, Artificial Sequence
  Primer-2 for rat CD68
cattcccttacggacagcttac

SEQ ID NO: 16 - DNA, 22 bp, Artificial Sequence
  Probe for human RPLP0
ccctgtcttccctgggcatcac

SEQ ID NO: 17 - DNA, 21 bp, Artificial Sequence
  Primer-1 for human RPLP0
tgtctgctcccacaatgaaac

SEQ ID NO: 18 - DNA, 20 bp, Artificial Sequence
  Primer-2 for human RPLP0
tcgtctttaaaccctgcgtg

SEQ ID NO: 19 - DNA, 25 bp, Artificial Sequence
  Probe for human CD68
aggtcctgcatgaatccaaagctga

SEQ ID NO: 20 - DNA, 22 bp, Artificial Sequence
  Primer-1 for human CD68
ccatgtagctcaggtagacaac

SEQ ID NO: 21 - DNA, 20 bp, Artificial Sequence
  Primer-2 for human CD68
ccacctgcttctctcattcc

SEQ ID NO: 22 - DNA, 24 bp, Artificial Sequence
  Probe for human CD163
atccatctgagcaggtcactccag

SEQ ID NO: 23 - DNA, 22 bp, Artificial Sequence
  Primer-1 for human CD163
ccagaacacatattccctccac

SEQ ID NO: 24 - DNA, 24 bp, Artificial Sequence
  Primer-2 for human CD163
gcatagtaactgtactcaccaaca

SEQ ID NO: 25 - DNA, 26 bp, Artificial Sequence
  Probe for human CD34
ccttgcaacatctcccactaaaccct

SEQ ID NO: 26 - DNA, 22 bp, Artificial Sequence
  Primer-1 for human CD34
tgcctgaacatttgatttctgc

SEQ ID NO: 27 - DNA, 21 bp, Artificial Sequence
  Primer-2 for human CD34
gacctttcaaccactagcact